European Patent Specification EP 3 677 590 B1, published March 27, 2024. Title: Peptides Having Activity for Wrinkle Relief and Uses Thereof. Applicant: CAREGEN CO., LTD. The sequence listing filed with the application follows.

SEQUENCE LISTING (16 sequences)

SEQ ID NO: 1 - protein, 7 aa, Artificial Sequence
  Peptide 1
KWGGGRY

SEQ ID NO: 2 - protein, 7 aa, Artificial Sequence
  Peptide 2
ILGRWCG

SEQ ID NO: 3 - protein, 4 aa, Artificial Sequence
  Peptide 3
GPVH

SEQ ID NO: 4 - protein, 11 aa, Artificial Sequence
  Peptide 4
EDEFKPPAAGR

SEQ ID NO: 5 - DNA, 20 bp, Artificial Sequence
  Collagen1a_F
caccctcaagagcctgagtc

SEQ ID NO: 6 - DNA, 20 bp, Artificial Sequence
  Collagen1a_R
agacggctgagtagggaaca

SEQ ID NO: 7 - DNA, 20 bp, Artificial Sequence
  Fibronectin_F
ccaggaaccgagtacaccat

SEQ ID NO: 8 - DNA, 20 bp, Artificial Sequence
  Fibronectin_R
atacccaggttgggtgatga

SEQ ID NO: 9 - DNA, 20 bp, Artificial Sequence
  Elastin_F
ggacccctgactcgcgacct

SEQ ID NO: 10 - DNA, 20 bp, Artificial Sequence
  Elastin_R
ggggaggtgggactgcccaa

SEQ ID NO: 11 - DNA, 25 bp, Artificial Sequence
  GAPDH_F
ggtgtgaacggatttggccgtattg

SEQ ID NO: 12 - DNA, 25 bp, Artificial Sequence
  GAPDH_R
ccgttgaatttgccgtgagtggagt

SEQ ID NO: 13 - DNA, 20 bp, Artificial Sequence
  AQP3_F
ccttcttgggtgctggaata

SEQ ID NO: 14 - DNA, 20 bp, Artificial Sequence
  AQP3_R
acacgataagggaggctctg

SEQ ID NO: 15 - DNA, 20 bp, Artificial Sequence
  SIRT1_F
tcagtggctggaacagtgag

SEQ ID NO: 16 - DNA, 20 bp, Artificial Sequence
  SIRT1_R
tctggcatgtcccactatca